European Patent Specification EP 3 730 612 B1, published February 4, 2026. Title: Immune cells expressing IL-7, CCL19, and cell surface molecules which specifically recognize human mesothelin. Applicant: YAMAGUCHI UNIVERSITY. The sequence listing filed with the application follows.

SEQUENCE LISTING (33 sequences)

SEQ ID NO: 1 - protein, 128 aa, artificial
  VH07_aa
  Inventor: Tamada, Koji; Sakoda, Yukimi; Adachi, Keishi
QVQLQQSGPGLVTPSQTLSLTCAISGDSVSSNSATWNWIRQSPSRGLEWLGRTYYRSKWYNDYAVSVKSRMSINPDTSKNQFSLQLNSVTPEDTAVYYCARGMMTYYYGMDVWGQGTTVTVSSGILGS

SEQ ID NO: 2 - protein, 116 aa, artificial
  VL07_aa
QPVLTQSSSLSASPGASASLTCTLRSGINVGPYRIYWYQQKPGSPPQYLLNYKSDSDKQQGSGVPSRFSGSKDASANAGVLLISGLRSEDEADYYCMIWHSSAAVFGGGTQLTVLS

SEQ ID NO: 3 - protein, 128 aa, artificial
  VH36_aa
QVQLQQSGPGLVTPSQTLSLTCAISGDSVSSNSATWNWIRQSPSRGLEWLGRTYYRSKWYNDYAVSVKSRMSINPDTSKNQFSLQLNSVTPEDTAVYYCARGMMTYYYGMDVWGQGTTVTVSSGILLS

SEQ ID NO: 4 - protein, 115 aa, artificial
  VL36_aa
QPVLTQSSSLSASPGASASLTCTLRSGINVGPRIYWYQQKPGSPPQYLLNYKSDSDKQQGSGVPSRFSGSKDASANAGVLLISGLRSEDEADYYCMIWHSSAAVFGGGTQLTVLS

SEQ ID NO: 5 - protein, 119 aa, artificial
  VHMO_aa
QVQLVQSGAEVKKPGASVKVSCKASGYTFTGNYINWVRQAPGQGLEWMGIINPTKGWTLYAQKFQGRVTMTRDTSISTAYMELSSLRSEDTAVYYCARWHHGTWIFDYWGQGTLVTVSS

SEQ ID NO: 6 - protein, 109 aa, artificial
  VLMO_aa
DIVLTQPPSVSGAPGQRVTISCSGSSSNIGSNYVSWYQQLPGTAPKLLIYNDNQRPSGVPDRFSGSKSGTSASLAITGLQSEDEADYYCSTYDRRTFSVFGGGTKLTVL

SEQ ID NO: 7 - protein, 21 aa, artificial
  CD8 M_aa
IYIWAPLAGTCGVLLLSLVIT

SEQ ID NO: 8 - protein, 41 aa, artificial
  CD28_A_aa
RSKRSRLLHSDYMNMTPRRPGPTRKHYQPYAPPRDFAAYRS

SEQ ID NO: 9 - protein, 46 aa, artificial
  4-1 BB_A_aa
RFSVVKRGRKKLLYIFKQPFMRPVQTTQEEDGCSCRFPEEEEGGCE

SEQ ID NO: 10 - protein, 113 aa, artificial
  CD3z_A_aa
LRVKFSRSADAPAYQQGQNQLYNELNLGRREEYDVLDKRRGRDPEMGGKPRRKNPQEGLYNELQKDKMAEAYSEIGMKGERRRGKGHDGLYQGLSTATKDTYDALHMQALPPR

SEQ ID NO: 11 - protein, 19 aa, artificial
  signal peptideT_aa
MDWTWRILFLVAAATGAHS

SEQ ID NO: 12 - protein, 23 aa, artificial
  signal peptide P_aa
MALPVTALLLPLALLLHAARPGS

SEQ ID NO: 13 - protein, 10 aa, artificial
  VH07_CDR1_aa
GDSVSSNSAT

SEQ ID NO: 14 - protein, 9 aa, artificial
  VH07_CDR2_aa
TYYRSKWYN

SEQ ID NO: 15 - protein, 13 aa, artificial
  VH07_CDR3_aa
ARGMMTYYYGMDV

SEQ ID NO: 16 - protein, 9 aa, artificial
  VL07_CDR1_aa
SGINVGPYR

SEQ ID NO: 17 - protein, 7 aa, artificial
  VL07_CDR2_aa
YKSDSDK

SEQ ID NO: 18 - protein, 9 aa, artificial
  VL07_CDR3_aa
MIWHSSAAV

SEQ ID NO: 19 - protein, 8 aa, artificial
  VL36_CDR1_aa
SGINVGPR

SEQ ID NO: 20 - protein, 8 aa, artificial
  VHMO_CDR1_aa
GYTFTGNY

SEQ ID NO: 21 - protein, 8 aa, artificial
  VHMO_CDR2_aa
INPTKGWT

SEQ ID NO: 22 - protein, 12 aa, artificial
  VHMO_CDR3_aa
ARWHHGTWIFDY

SEQ ID NO: 23 - protein, 8 aa, artificial
  VLMO_CDR1_aa
SSNIGSNY

SEQ ID NO: 24 - protein, 3 aa, artificial
  VLMO_CDR2_aa
NDN

SEQ ID NO: 25 - protein, 10 aa, artificial
  VLMO_CDR3_aa
STYDRRTFSV

SEQ ID NO: 26 - protein, 15 aa, artificial
  linker 15_aa
GGGGSGGGGSGGGGS

SEQ ID NO: 27 - protein, 25 aa, artificial
  linker 25_aa
SSADDAKKDAAKKDDAKKDDAKKDG

SEQ ID NO: 28 - protein, 177 aa, Homo sapiens
MFHVSFRYIFGLPPLILVLLPVASSDCDIEGKDGKQYESVLMVSIDQLLDSMKEIGSNCLNNEFNFFKRHICDANKEGMFLFRAARKLRQFLKMNSTGDFDLHLLKVSEGTTILLNCTGQVKGRKPAALGEAQPTKSLEENKSLKEQKKLNDLCFLKRLLQEIKTCWNKILMGTKEH

SEQ ID NO: 29 - protein, 98 aa, Homo sapiens
MALLLALSLLVLWTSPAPTLSGTNDAEDCCLSVTQKPIPGYIVRNFHYLLIKDGCRVPAVVFTTLRGRQLCAPPDQPWVERIIQRLQRTSAKMKRRSS

SEQ ID NO: 30 - DNA, 531 bp, Homo sapiens
atgttccatgtttcttttaggtatatctttggacttcctcccctgatccttgttctgttgccagtagcatcatctgattgtgatattgaaggtaaagatggcaaacaatatgagagtgttctaatggtcagcatcgatcaattattggacagcatgaaagaaattggtagcaattgcctgaataatgaatttaacttttttaaaagacatatctgtgatgctaataaggaaggtatgtttttattccgtgctgctcgcaagttgaggcaatttcttaaaatgaatagcactggtgattttgatctccacttattaaaagtttcagaaggcacaacaatactgttgaactgcactggccaggttaaaggaagaaaaccagctgccctgggtgaagcccaaccaacaaagagtttggaagaaaataaatctttaaaggaacagaaaaaactgaatgacttgtgtttcctaaagagactattacaagagataaaaacttgttggaataaaattttgatgggcactaaagaacac

SEQ ID NO: 31 - DNA, 294 bp, Homo sapiens
atggccctgctactggccctcagcctgctggttctctggacttccccagccccaactctgagtggcaccaatgatgctgaagactgctgcctgtctgtgacccagaaacccatccctgggtacatcgtgaggaacttccactaccttctcatcaaggatggctgcagggtgcctgctgtagtgttcaccacactgaggggccgccagctctgtgcacccccagaccagccctgggtagaacgcatcatccagagactgcagaggacctcagccaagatgaagcgccgcagcagt

SEQ ID NO: 32 - protein, 8 aa, artificial
  2A peptide cleavage region
  MISC_FEATURE (2)..(2): Val or Ile
  MISC_FEATURE (4)..(4): any amino acid
DXEXNPGP

SEQ ID NO: 33 - protein, 25 aa, artificial
  F2A_aa
GSGVKQTLNFDLLKLAGDVESNPGP